European Patent Application EP 4 438 732 A1, published October 2, 2024. Title: Novel promoter variant for constitutive expression and use of the same. Applicant: DAESANG CORPORATION. Application WO. The sequence listing filed with the application follows.

SEQUENCE LISTING (26 sequences)

SEQ ID NO: 1 - DNA, 160 bp, Escherichia coli
  source 1..160: mol_type = genomic DNA
acctgaatgggggttgatgcccggctggttaatggcaggtggtctgatcgcctggtttgtcggttggcgcaaaacacgctgattttttcatcgctcaaggcgggccgtgtaacgtataatgcggctttgtttaatcatcatctaccacagaggaacatgt

SEQ ID NO: 2 - DNA, 115 bp, Bacillus licheniformis
  source 1..115: mol_type = genomic DNA
ggtgtctcattctgttaccgttaacagctgaaaatgattgttcctgttaccgccgtcatgataatttcagaataaaagccggtttatcacagccggacaaccaaaagggggaaac

SEQ ID NO: 3 - protein, 294 aa, Flavonifractor plautii
MNPIGMHYGFWSHNWDEIAYIPLMEKLAWLGFDICEVASAEWGYYDDARLRELKACADHNGLGITYSIGLEAKYDLASDDPAVRENGIRHVTRILESMPKVGAAILNGVSYAGWQALPDHGITLDEKRRKEELALESMSRLMKVAEDCGVLYCCEVVNRFEQYLLNTAKEGVEFVKRLGSPNARVLLDTFHMNIEEDSMVDAILEAGPWLGHFHVGENNRRPAGSTNRLPWKDMAAALKQVNYQGAIVMEPFVLMGGTIPYDIKVWRDLSGGAGEAGLDEMAGRACRFLKELTA

SEQ ID NO: 4 - DNA, 885 bp, Flavonifractor plautii
  source 1..885: mol_type = genomic DNA
atgaacccgattggaatgcactacggcttctggagccacaactgggacgagattgcatacatacccctgatggagaagctggcctggctgggctttgacatctgcgaggtggcctccgccgagtggggctattacgacgacgccaggctgcgggagctgaaggcctgcgccgatcacaacggcctgggcatcacctattccatcggcctggaggccaaatacgacctggccagcgacgatccggcggtgcgggagaacggcatccgccatgtcacccgcatcctggagagcatgcccaaggtgggggcggccatcctcaacggcgtgtcctacgccgggtggcaggccctgcccgaccacggaatcaccctggacgagaagcgccgcaaggaggagcttgccctggagtccatgtcccggctcatgaaggtggcggaggactgcggcgtgctctactgctgcgaggtggtcaaccgcttcgagcagtacctgctcaacaccgccaaagagggcgtggagtttgtcaagcgcctgggcagtcccaacgcccgggtgctgctggataccttccacatgaacatcgaggaggacagcatggtggacgccattctggaggcgggcccctggctggggcatttccacgtgggggagaacaaccgccgccccgccggctccaccaaccgcctgccctggaaggacatggccgccgccctcaagcaggtgaactaccagggggccattgtgatggagcccttcgtgctcatggggggtaccattccctatgatatcaaggtctggcgggatctcagcggcggggccggggaggccgggctggacgagatggcgggccgggcctgccggttcctcaaggagctgaccgcgtaa

SEQ ID NO: 5 - protein, 294 aa, synthetic construct
MNPIGMHYGFWSHNWDEIAYIPLMEKLAKLGFDICEVASAEWGYYDDARLRELKACADHNGLGITYSIGLEAKYDLASDDPAVRENGIRHVTRILESMPKVGAAILNGVSYAGWQALPDHGITLDEKRRKEELALESMSRLMKVAEDCGVLYCCEVVNRFEQYLLNTAKEGVEFVKRLGSPNARVLLDTFHMNIEEDSMVDAILEAGPWLGHFHVSENNRRPAGSTNRLPWKDIAAALKQVNYQGAIVMEPFVLMGGTIPYDIKVWRDLSGGAGEAGLDEMAGRACRFLKELTA

SEQ ID NO: 6 - DNA, 885 bp, synthetic construct
  source 1..885: mol_type = other DNA
atgaacccgattggaatgcactacggcttctggagccacaactgggacgagattgcatacatacccctgatggagaagctggccaaactgggctttgacatctgcgaggtggcctccgccgagtggggctattacgacgacgccaggctgcgggagctgaaggcctgcgccgatcacaacggcctgggcatcacctattccatcggcctggaggccaaatacgacctggccagcgacgatccggcggtgcgggagaacggcatccgccatgtcacccgcatcctggagagcatgcccaaggtgggggcggccatcctcaacggcgtgtcctacgccgggtggcaggccctgcccgaccacggaatcaccctggacgagaagcgccgcaaggaggagcttgccctggagtccatgtcccggctcatgaaggtggcggaggactgcggcgtgctctactgctgcgaggtggtcaaccgcttcgagcagtacctgctcaacaccgccaaagagggcgtggagtttgtcaagcgcctgggcagtcccaacgcccgggtgctgctggataccttccacatgaacatcgaggaggacagcatggtggacgccattctggaggcgggcccctggctggggcatttccacgtgagcgagaacaaccgccgccccgccggctccaccaaccgcctgccctggaaggacattgccgccgccctcaagcaggtgaactaccagggggccattgtgatggagcccttcgtgctcatggggggtaccattccctatgatatcaaggtctggcgggatctcagcggcggggccggggaggccgggctggacgagatggcgggccgggcctgccggttcctcaaggagctgaccgcgtaa

SEQ ID NO: 7 - protein, 294 aa, synthetic construct
MNPIGMHYGFWSHNWDEIAYIPLMEKLAKLGFDICEVASAEWGYYDDARLRELKACADHNGLGITYSIGLEAKYDLSSDDPAVRENGIRHVTRILESMPKVGAAILNGVSYAGWQALPDHGITLDEKRRKEELALESMSRLMKVAEDCGVLYCCEVVNRFEQYLLNTAKEGVEFVKRLGSPNARVLLDTFHMNIEEDSMVDAILEAGPWLGHFHVSENNRRPAGSTNRLPWKDIAAALKQVNYQGAIVMEPFVLMGGTIPYDIKVWRDLSGGAGEAGLDEMAGRACRFLKELTA

SEQ ID NO: 8 - DNA, 885 bp, synthetic construct
  source 1..885: mol_type = other DNA
atgaacccgattggaatgcactacggcttctggagccacaactgggacgagattgcatacatacccctgatggagaagctggccaaactgggctttgacatctgcgaggtggcctccgccgagtggggctattacgacgacgccaggctgcgggagctgaaggcctgcgccgatcacaacggcctgggcatcacctattccatcggcctggaggccaaatacgacctgagcagcgacgatccggcggtgcgggagaacggcatccgccatgtcacccgcatcctggagagcatgcccaaggtgggggcggccatcctcaacggcgtgtcctacgccgggtggcaggccctgcccgaccacggaatcaccctggacgagaagcgccgcaaggaggagcttgccctggagtccatgtcccggctcatgaaggtggcggaggactgcggcgtgctctactgctgcgaggtggtcaaccgcttcgagcagtacctgctcaacaccgccaaagagggcgtggagtttgtcaagcgcctgggcagtcccaacgcccgggtgctgctggataccttccacatgaacatcgaggaggacagcatggtggacgccattctggaggcgggcccctggctggggcatttccacgtgagcgagaacaaccgccgccccgccggctccaccaaccgcctgccctggaaggacattgccgccgccctcaagcaggtgaactaccagggggccattgtgatggagcccttcgtgctcatggggggtaccattccctatgatatcaaggtctggcgggatctcagcggcggggccggggaggccgggctggacgagatggcgggccgggcctgccggttcctcaaggagctgaccgcgtaa

SEQ ID NO: 9 - DNA, 161 bp, synthetic construct
  source 1..161: mol_type = other DNA
acctgaatgggggttgatgcccggctggttaatggcaggtggtctgatcgcctggtttgtcggttggcgcaaaacacgctgattttttcatcgctcaaggcgggccgtgtaacgtataatgcggctttgtttaatcatcatctaccacagaggaacatgtc

SEQ ID NO: 10 - DNA, 158 bp, synthetic construct
  source 1..158: mol_type = other DNA
acctgaatgggggttgatgcccggctggttaatggcaggtggtctgatcgcctggtttgtcggttggcgcaaaacacgctgattttttcatcgctcaaggcgggccgtgtaacgtataatgcggctttgtttaatcatcatctacgaaggaggaacat

SEQ ID NO: 11 - DNA, 20 bp, synthetic construct
  source 1..20: mol_type = other DNA
acctgaatgggggttgatgc

SEQ ID NO: 12 - DNA, 19 bp, synthetic construct
  source 1..19: mol_type = other DNA
acatgttcctctgtggtag

SEQ ID NO: 13 - DNA, 20 bp, synthetic construct
  source 1..20: mol_type = other DNA
ggtgtctcattctgttaccg

SEQ ID NO: 14 - DNA, 20 bp, synthetic construct
  source 1..20: mol_type = other DNA
gtttcccccttttggttgtc

SEQ ID NO: 15 - DNA, 32 bp, synthetic construct
  source 1..32: mol_type = other DNA
aatacgacctgagcagcgacgatccggcggtg

SEQ ID NO: 16 - DNA, 33 bp, synthetic construct
  source 1..33: mol_type = other DNA
gatcgtcgctgctcaggtcgtatttggcctcca

SEQ ID NO: 17 - DNA, 29 bp, synthetic construct
  source 1..29: mol_type = other DNA
gcatgccatatgaacccgattggaatgca

SEQ ID NO: 18 - DNA, 32 bp, synthetic construct
  source 1..32: mol_type = other DNA
gcatgcctcgagcgcggtcagctccttgagga

SEQ ID NO: 19 - DNA, 32 bp, synthetic construct
  source 1..32: mol_type = other DNA
tttgcgctcgagacctgaatgggggttgatgc

SEQ ID NO: 20 - DNA, 39 bp, synthetic construct
  source 1..39: mol_type = other DNA
tgcattccaatcgggttcatacatgttcctctgtggtag

SEQ ID NO: 21 - DNA, 39 bp, synthetic construct
  source 1..39: mol_type = other DNA
ctaccacagaggaacatgtatgaacccgattggaatgca

SEQ ID NO: 22 - DNA, 31 bp, synthetic construct
  source 1..31: mol_type = other DNA
gcatgctgcagttacgcggtcagctccttga

SEQ ID NO: 23 - DNA, 32 bp, synthetic construct
  source 1..32: mol_type = other DNA
tttgcgctcgagggtgtctcattctgttaccg

SEQ ID NO: 24 - DNA, 40 bp, synthetic construct
  source 1..40: mol_type = other DNA
tgcattccaatcgggttcatgtttcccccttttggttgtc

SEQ ID NO: 25 - DNA, 40 bp, synthetic construct
  source 1..40: mol_type = other DNA
gacaaccaaaagggggaaacatgaacccgattggaatgca

SEQ ID NO: 26 - DNA, 31 bp, synthetic construct; identical to SEQ ID NO: 22
  source 1..31: mol_type = other DNA